European Patent Application EP 4 406 563 A1, published July 31, 2024. Title: MODIFIED SIS MEMBRANE FOR TISSUE REPAIR, PREPARATION METHOD THEREFOR, AND USE THEREOF. Applicant: BEIJING BIOSIS HEALING BIOLOGICAL TECHNOLOGY CO., LTD. The sequence listing filed with the application follows.

SEQUENCE LISTING (18 sequences)

SEQ ID NO: 1 - protein, 9 aa, Artificial Sequence
  collagen-binding peptide I
LHERHLNNN

SEQ ID NO: 2 - protein, 7 aa, Artificial Sequence
  collagen-binding peptide III
KELNLVY

SEQ ID NO: 3 - protein, 5 aa, Artificial Sequence
  linker peptide
GGGGS

SEQ ID NO: 4 - protein, 12 aa, Artificial Sequence
  polypeptide CP05
CRHSQMTVTSRL

SEQ ID NO: 5 - protein, 26 aa, Artificial Sequence
  polypeptide Pep1
LHERHLNNNGGGGSCRHSQMTVTSRL

SEQ ID NO: 6 - protein, 24 aa, Artificial Sequence
  polypeptide Pep2
KELNLVYGGGGSCRHSQMTVTSRL

SEQ ID NO: 7 - protein, 21 aa, Artificial Sequence
  polypeptide Pep3
LHERHLNNNCRHSQMTVTSRL

SEQ ID NO: 8 - protein, 19 aa, Artificial Sequence
  polypeptide Pep4
KELNLVYCRHSQMTVTSRL

SEQ ID NO: 9 - DNA, 21 bp, Artificial Sequence
  primer sequence
agttgtgcggaggtgatgtat

SEQ ID NO: 10 - DNA, 21 bp, Artificial Sequence
  primer sequence
ccggatgatagcaggctgtag

SEQ ID NO: 11 - DNA, 20 bp, Artificial Sequence
  primer sequence
gagcgactcggcagataagc

SEQ ID NO: 12 - DNA, 20 bp, Artificial Sequence
  primer sequence
ccacacggcggatagatagc

SEQ ID NO: 13 - DNA, 22 bp, Artificial Sequence
  primer sequence
taaggtctgcgctaaacaactc

SEQ ID NO: 14 - DNA, 20 bp, Artificial Sequence
  primer sequence
cagatccctttcagagcggt

SEQ ID NO: 15 - DNA, 20 bp, Artificial Sequence
  primer sequence
gaggctggcttcatccactg

SEQ ID NO: 16 - DNA, 21 bp, Artificial Sequence
  primer sequence
atgctcctctatcgggttgtc

SEQ ID NO: 17 - DNA, 21 bp, Artificial Sequence
  primer sequence
aggtcggtgtgaacggatttg

SEQ ID NO: 18 - DNA, 19 bp, Artificial Sequence
  primer sequence
ggggtcgttgatggcaaca